European Patent Specification EP 3 381 934 B1, published May 31, 2023. Title: Protein for neutralizing programmed necrocytosis promotion antibody, and application of protein. Applicant: JIANG, Shisong LU, Wenshu. The sequence listing filed with the application follows.

SEQUENCE LISTING (11 sequences)

SEQ ID NO: 1 - protein, 233 aa, Homo sapiens
MSTESMIRDVELAEEALPKKTGGPQGSRRCLFLSLFSFLIVAGATTLFCLLHFGVIGPQREEFPRDLSLISPLAQAVRSSSRTPSDKPVAHVVANPQAEGQLQWLNRRANALLANGVELRDNQLVVPSEGLYLIYSQVLFKGQGCPSTHVLLTHTISRIAVSYQTKVNLLSAIKSPCQRETPEGAEAKPWYEPIYLGGVFQLEKGDRLSAEINRPDYLDFAESGQVYFGIIAL

SEQ ID NO: 2 - protein, 157 aa, Artificial sequence
  Polypeptide
VRSSSRTPSDKPVAHVVANPQAEGQLQWLNRRANALLANGVELRDNQLVVPSEGLYLIYSQVLFKGQGCPSTHVLLTHTISRIAVFHQTKVNLLSAIKSPCQRETPEGAEAKPWYEPIYLGGVFQLEKGDRLSAEINRPDYLDFAESGQVYFGIIAL

SEQ ID NO: 3 - protein, 80 aa, Artificial sequence
  Polypeptide
QLQWLNRRANALLANGVELRDNQLVVPSEGLYLIYSQVLFKGQGCPSTHVLLTHTISRIAVSYQTKVNLLSAIKSPCQRE

SEQ ID NO: 4 - protein, 80 aa, Artificial sequence
  Polypeptide
QLQWLNRRANALLANGVELRDNQLVVPSEGLYLIYSQVLFKGQGCPSTHVLLTHTISRIAVFHQTKVNLLSAIKSPCQRE

SEQ ID NO: 5 - protein, 10 aa, Aritificial sequence
  Polypeptide
RDNQLVVPSE

SEQ ID NO: 6 - protein, 10 aa, Aritificial sequence
  Polypeptide
DNQLVVPSEG

SEQ ID NO: 7 - protein, 10 aa, Artificial sequence
  Polypeptide
NQLVVPSEGL

SEQ ID NO: 8 - protein, 10 aa, Artificial sequence
  Polypeptide
QLVVPSEGLY

SEQ ID NO: 9 - protein, 214 aa, Homo sapiens
DIQMTQSPASLSASVGETVTITCRASGNIHIYLAWYQQKQGKSPQLLVYNAKTLADGVPSRFSGSGSGTQYSLKINSLQPEDFGSYYCQHFWSIPWTFGGGTKLEIKRADAAPTVSIFPPSSEQLTSGGASVVCFLNNFYPKDINVKWKIDGSERQNGVLNSWTDQDSKDSTYSMSSTLTLTKDEYERHNSYTCEATHKTSTSPIVKSFNRNEC

SEQ ID NO: 10 - protein, 454 aa, Homo sapiens
QIQLVQSGPELKKPGETVKISCKASGYTFTNYGMNWVKQAPGKGLKWMGWINTYTGEPTYADDFKGRFAFSLETSANTAYLQINNLRNEGMATYFCARHYRYAWFPYWGQGTLVTVSAAKTTPPSVYPLAPGCGDTTGSSVTLGCLVKGYFPESVTVTWNSGSLSSSVHTFPALLQSGLYTMSSSVTVPSSTWPSQTVTCSVAHPASSTTVDKKLEPSGPISTINPCPPCKECHKCPAPNLEGGPSVFIFPPNIKDVLMISLTPKVTCVVVDVSEDDPDVQISWFVNNVEVHTAQTQTHREDYNSTIRVVSTLPIQHQDWMSGKEFKCKVNNKDLPSPIERTISKIKGLVRAPQVYILPPPAEQLSRKDVSLTCLVVGFNPGDISVEWASNGHTEENYKDTAPVLDSDGSYFIYSKLNMKTSKWEKTDSFSCNVRHEGLKNYYLKKTISRSPGK

SEQ ID NO: 11 - protein, 7 aa, Homo sapiens
QLVVPSE